European Patent Application EP 4 397 747 A1, published July 10, 2024. Title: 高抗紫外辐射球孢白僵菌菌株及其定向诱变方法和用途. Applicant: 浙江泰达作物科技有限公司. Application CN. The sequence listing filed with the application follows.

SEQUENCE LISTING (1 sequence)

SEQ ID NO: 1 - DNA, 500 bp, Beauveria bassiana
  source 1..500: mol_type = other DNA
acctacctatcgttgcttcggcggactcgccccagcccggacgcggactggaccagcggcccgccggggacctcaaactcttgtattccagcatcttctgaatacgccgcaaggcaaaacaaatgaatcaaaactttcaacaacggatctcttggctctggcatcgatgaagaacgcagcgaaacgcgataagtaatgtgaattgcagaatccagtgaatcatcgaatctttgaacgcacattgcgcccgccagcattctggcgggcatgcctgttcgagcgtcatttcaaccctcgacctccccttggggaggtcggcgttggggaccggcagcacaccgccggccctgaaatggagtggcggcccgtccgcggcgacctctgcgcagtaatacagctcgcaccggaaccccgacgcggccacgccgtaaaacacccaacttctgaacgttgacctcgaatcaggtaggactacccgctgaacttaagcatatcaataa